European Patent Application EP 4 144 848 A1, published March 8, 2023. Title: Novel L-tyrosine exporter variant and the method of producing L-tyrosine using the same. Applicant: CJ CheilJedang Corporation. The sequence listing filed with the application follows.

SEQUENCE LISTING (85 sequences)

SEQ ID NO: 1 - protein, 307 aa, Artificial Sequence
  Wex L79A
MNSKKATLIGLTAVVLWSSIVGLIRGVSEHLGATGGAAMMYSVASLFLLLSVGFPKLGSFPKKYLLWGSLLFVSYELCASLSIGYANTGRQAIEVSMVNYLWPAFTLIAAIAFNRQRANWMVVPGFILSIIGICWVLGGDQGLDLAGMLGNVQDNPLSYGLAFLGAVIWAAYCTVTARLAKGKNGVTLFFILVALTLWVKFFFGDHRPMSFSLPAIVYLLLAAAAMGFGYAAWNVGILHGNVTVLAGVSYFIPVFSAALSAMVLHAPLPRSFWVGASLVCAGSILCWLATRARRASAAQEDAVADCL

SEQ ID NO: 2 - protein, 307 aa, Artificial Sequence
  Wex L79G
MNSKKATLIGLTAVVLWSSIVGLIRGVSEHLGATGGAAMMYSVASLFLLLSVGFPKLGSFPKKYLLWGSLLFVSYELCGSLSIGYANTGRQAIEVSMVNYLWPAFTLIAAIAFNRQRANWMVVPGFILSIIGICWVLGGDQGLDLAGMLGNVQDNPLSYGLAFLGAVIWAAYCTVTARLAKGKNGVTLFFILVALTLWVKFFFGDHRPMSFSLPAIVYLLLAAAAMGFGYAAWNVGILHGNVTVLAGVSYFIPVFSAALSAMVLHAPLPRSFWVGASLVCAGSILCWLATRARRASAAQEDAVADCL

SEQ ID NO: 3 - DNA, 35 bp, Artificial Sequence
  primer
tcgagctcggtaccctgggaacttgtcgacgctat

SEQ ID NO: 4 - DNA, 35 bp, Artificial Sequence
  primer
tgttcggcaagcattgtggtgtgggcaatgatcac

SEQ ID NO: 5 - DNA, 35 bp, Artificial Sequence
  primer
attaacggttaaagtactcattgtgaggtggcggg

SEQ ID NO: 6 - DNA, 35 bp, Artificial Sequence
  primer
ctctagaggatccccggagctgctgtccaacgtgg

SEQ ID NO: 7 - DNA, 35 bp, Artificial Sequence
  primer
ccacaccacaatgcttgccgaacatttttcttttc

SEQ ID NO: 8 - DNA, 35 bp, Artificial Sequence
  primer
cacaatgagtactttaaccgttaatggagtccttg

SEQ ID NO: 9 - DNA, 17 bp, Artificial Sequence
  primer
acgcgccaagtcggacg

SEQ ID NO: 10 - DNA, 19 bp, Artificial Sequence
  primer
cgcacgatgtttacctgcg

SEQ ID NO: 11 - DNA, 1122 bp, Artificial Sequence
  E.coli tyrA_M53I_A354V
atggttgctgaattgaccgcattacgcgatcaaattgatgaagtcgataaagcgctgctgaatttattagcgaagcgtctggaactggttgctgaagtgggcgaggtgaaaagccgctttggactgcctatttatgttccggagcgcgaggcatctattttggcctcgcgtcgtgcagaggcggaagctctgggtgtaccgccagatctgattgaggatgttttgcgtcgggtgatgcgtgaatcttactccagtgaaaacgacaaaggatttaaaacactttgtccgtcactgcgtccggtggttatcgtcggcggtggcggtcagatgggacgcctgttcgagaagatgctgaccctctcgggttatcaggtgcggattctggagcaacatgactgggatcgagcggctgatattgttgccgatgccggaatggtgattgttagtgtgccaatccacgttactgagcaagttattggcaaattaccgcctttaccgaaagattgtattctggtcgatctggcatcagtgaaaaatgggccattacaggccatgctggtggcgcatgatggtccggtgctggggctacacccgatgttcggtccggacagcggtagcctggcaaagcaagttgtggtctggtgtgatggacgtaaaccggaagcataccaatggtttctggagcaaattcaggtctggggcgctcggctgcatcgtattagcgccgtcgagcacgatcagaatatggcgtttattcaggcactgcgccactttgctacttttgcttacgggctgcacctggcagaagaaaatgttcagcttgagcaacttctggcgctctcttcgccgatttaccgccttgagctggcgatggtcgggcgactgtttgctcaggatccgcagctttatgccgacatcattatgtcgtcagagcgtaatctggcgttaatcaaacgttactataagcgtttcggcgaggcgattgagttgctggagcagggcgataagcaggcgtttattgacagtttccgcaaggtggagcactggttcggcgattacgtgcagcgttttcagagtgaaagccgcgtgttattgcgtcaggcgaatgacaatcgccagtaa

SEQ ID NO: 12 - DNA, 36 bp, Artificial Sequence
  primer
ttcgagctcggtaccctatcaaaaccgagttcttcc

SEQ ID NO: 13 - DNA, 36 bp, Artificial Sequence
  primer
gtcgtttttaggcctcctgacaagtgtggcacatac

SEQ ID NO: 14 - DNA, 36 bp, Artificial Sequence
  primer
tgacaatcgccagtaattttatcggctgatgattct

SEQ ID NO: 15 - DNA, 36 bp, Artificial Sequence
  primer
actctagaggatccccaacgcgattgcattcggctc

SEQ ID NO: 16 - DNA, 36 bp, Artificial Sequence
  primer
gtgccacacttgtcaggaggcctaaaaacgaccgag

SEQ ID NO: 17 - DNA, 36 bp, Artificial Sequence
  primer
tcaattcagcaaccatgttgtgtctcctctaaagat

SEQ ID NO: 18 - DNA, 36 bp, Artificial Sequence
  primer
ttagaggagacacaacatggttgctgaattgaccgc

SEQ ID NO: 19 - DNA, 36 bp, Artificial Sequence
  primer
tcatcagccgataaaattactggcgattgtcattcg

SEQ ID NO: 20 - DNA, 18 bp, Artificial Sequence
  primer
gcccactagtcgaatccc

SEQ ID NO: 21 - DNA, 18 bp, Artificial Sequence
  primer
ctgtccgcaacctgtgcg

SEQ ID NO: 22 - DNA, 1053 bp, Artificial Sequence
  E.coli aroG_P150L
atgaattatcagaacgacgatttacgcatcaaagaaatcaaagagttacttcctcctgtcgcattgctggaaaaattccccgctactgaaaatgccgcgaatacggttgcccatgcccgaaaagcgatccataagatcctgaaaggtaatgatgatcgcctgttggttgtgattggcccatgctcaattcatgatcctgtcgcggcaaaagagtatgccactcgcttgctggcgctgcgtgaagagctgaaagatgagctggaaatcgtaatgcgcgtctattttgaaaagccgcgtaccacggtgggctggaaagggctgattaacgatccgcatatggataatagcttccagatcaacgacggtctgcgtatagcccgtaaattgctgcttgatattaacgacagcggtctgccagcggcaggtgagtttctcgatatgatcaccccacaatatctcgctgacctgatgagctggggcgcaattggcgcacgtaccaccgaatcgcaggtgcaccgcgaactggcatcagggctttcttgtccggtcggcttcaaaaatggcaccgacggtacgattaaagtggctatcgatgccattaatgccgccggtgcgccgcactgcttcctgtccgtaacgaaatgggggcattcggcgattgtgaataccagcggtaacggcgattgccatatcattctgcgcggcggtaaagagcctaactacagcgcgaagcacgttgctgaagtgaaagaagggctgaacaaagcaggcctgccagcacaggtgatgatcgatttcagccatgctaactcgtccaaacaattcaaaaagcagatggatgtttgtgctgacgtttgccagcagattgccggtggcgaaaaggccattattggcgtgatggtggaaagccatctggtggaaggcaatcagagcctcgagagcggggagccgctggcctacggtaagagcatcaccgatgcctgcatcggctgggaagataccgatgctctgttacgtcaactggcgaatgcagtaaaagcgcgtcgcgggtaa

SEQ ID NO: 23 - DNA, 35 bp, Artificial Sequence
  primer
tcgagctcggtaccccccggcggtatcgaggtagt

SEQ ID NO: 24 - DNA, 35 bp, Artificial Sequence
  primer
gacaagtttagtactttaatcacccgcggggaccc

SEQ ID NO: 25 - DNA, 35 bp, Artificial Sequence
  primer
ggtgattaaagtactaaacttgtcccgagggtgag

SEQ ID NO: 26 - DNA, 35 bp, Artificial Sequence
  primer
ctctagaggatcccctatcagtcacttccctgaga

SEQ ID NO: 27 - DNA, 35 bp, Artificial Sequence
  primer
gcgggtgattaaagtgaggcctaaaaacgaccgag

SEQ ID NO: 28 - DNA, 35 bp, Artificial Sequence
  primer
gttctgataattcatgttgtgtctcctctaaagat

SEQ ID NO: 29 - DNA, 20 bp, Artificial Sequence
  primer
atgaattatcagaacgacga

SEQ ID NO: 30 - DNA, 35 bp, Artificial Sequence
  primer
cgggacaagtttagtttacccgcgacgcgctttta

SEQ ID NO: 31 - DNA, 20 bp, Artificial Sequence
  primer
ttgatatgaccgcagcctga

SEQ ID NO: 32 - DNA, 20 bp, Artificial Sequence
  primer
ctgcattctcatcgatcttg

SEQ ID NO: 33 - DNA, 34 bp, Artificial Sequence
  primer
ttcgagctcggtacccggaggggtttccacctcg

SEQ ID NO: 34 - DNA, 40 bp, Artificial Sequence
  primer
tgggaagcttgtctcaattatgtctgttgctcaattagcg

SEQ ID NO: 35 - DNA, 38 bp, Artificial Sequence
  primer
ctaattgagcaacagacataattgagacaagcttccca

SEQ ID NO: 36 - DNA, 36 bp, Artificial Sequence
  primer
aattggtgcgtcgctcatggggcacctaccgaggaa

SEQ ID NO: 37 - DNA, 40 bp, Artificial Sequence
  primer
ttcctcggtaggtgccccatgagcgacgcaccaattgttg

SEQ ID NO: 38 - DNA, 36 bp, Artificial Sequence
  primer
cgactctagaggatccccccgaagagttcggctgcg

SEQ ID NO: 39 - DNA, 18 bp, Artificial Sequence
  primer
ccagcgatgatcgcgccg

SEQ ID NO: 40 - DNA, 18 bp, Artificial Sequence
  primer
atcgccgtggagccagcc

SEQ ID NO: 41 - DNA, 35 bp, Artificial Sequence
  primer
ttcgagctcggtacccgagggctcactgacgttga

SEQ ID NO: 42 - DNA, 34 bp, Artificial Sequence
  primer
cgctgggatgtttctaccggattcgattcctcag

SEQ ID NO: 43 - DNA, 35 bp, Artificial Sequence
  primer
cgctcccagaagtaggctcaaaccttgcccataac

SEQ ID NO: 44 - DNA, 35 bp, Artificial Sequence
  primer
ctctagaggatccccctcccccaaaccacgctttt

SEQ ID NO: 45 - DNA, 318 bp, Artificial Sequence
  CJ7 promoter
agaaacatcccagcgctactaatagggagcgttgaccttccttccacggaccggtaatcggagtgcctaaaaccgcatgcggcttaggctccaagataggttctgcgcggccgggtaatgcatcttctttagcaacaagttgaggggtaggtgcaaataagaacgacatagaaatcgtctcctttctgtttttaatcaacatacaccaccacctaaaaattccccgaccagcaagttcacagtattcgggcacaatatcgttgccaaaatattgtttcggaatatcatgggatacgtacccaacgaaaggaaacactc

SEQ ID NO: 46 - DNA, 35 bp, Artificial Sequence
  primer
ggaatcgaatccggtagaaacatcccagcgctact

SEQ ID NO: 47 - DNA, 35 bp, Artificial Sequence
  primer
tactttcagaactcatgagtgtttcctttcgttgg

SEQ ID NO: 48 - DNA, 35 bp, Artificial Sequence
  primer
acgaaaggaaacactcatgagttctgaaagtagtc

SEQ ID NO: 49 - DNA, 35 bp, Artificial Sequence
  primer
gggcaaggtttgagcctacttctgggagcgccaca

SEQ ID NO: 50 - DNA, 21 bp, Artificial Sequence
  primer
acattaagtggtaggcgctga

SEQ ID NO: 51 - DNA, 20 bp, Artificial Sequence
  primer
cataacagggcagaacaaac

SEQ ID NO: 52 - protein, 307 aa, Artificial Sequence
  wex AA seq
MNSKKATLIGLTAVVLWSSIVGLIRGVSEHLGATGGAAMMYSVASLFLLLSVGFPKLGSFPKKYLLWGSLLFVSYELCLSLSIGYANTGRQAIEVSMVNYLWPAFTLIAAIAFNRQRANWMVVPGFILSIIGICWVLGGDQGLDLAGMLGNVQDNPLSYGLAFLGAVIWAAYCTVTARLAKGKNGVTLFFILVALTLWVKFFFGDHRPMSFSLPAIVYLLLAAAAMGFGYAAWNVGILHGNVTVLAGVSYFIPVFSAALSAMVLHAPLPRSFWVGASLVCAGSILCWLATRARRASAAQEDAVADCL

SEQ ID NO: 53 - DNA, 20 bp, Artificial Sequence
  primer
cggattatgccaatgatgtg

SEQ ID NO: 54 - DNA, 20 bp, Artificial Sequence
  primer
cacgatcaccaacattcagg

SEQ ID NO: 55 - DNA, 40 bp, Artificial Sequence
  primer
gtgtcctacgaactctgcgcatcgctctccatcggttatg

SEQ ID NO: 56 - DNA, 40 bp, Artificial Sequence
  primer
cataaccgatggagagcgatgcgcagagttcgtaggacac

SEQ ID NO: 57 - DNA, 40 bp, Artificial Sequence
  primer
gtgtcctacgaactctgcatctcgctctccatcggttatg

SEQ ID NO: 58 - DNA, 40 bp, Artificial Sequence
  primer
cataaccgatggagagcgagatgcagagttcgtaggacac

SEQ ID NO: 59 - DNA, 37 bp, Artificial Sequence
  primer
gtgtcctacgaactctgcggctcgctctccatcggtt

SEQ ID NO: 60 - DNA, 36 bp, Artificial Sequence
  primer
cataaccgatggagagcgagccgcagagttcgtagg

SEQ ID NO: 61 - DNA, 37 bp, Artificial Sequence
  primer
gtgtcctacgaactctgcatgtcgctctccatcggtt

SEQ ID NO: 62 - DNA, 36 bp, Artificial Sequence
  primer
cataaccgatggagagcgacatgcagagttcgtagg

SEQ ID NO: 63 - DNA, 37 bp, Artificial Sequence
  primer
gtgtcctacgaactctgcacctcgctctccatcggtt

SEQ ID NO: 64 - DNA, 36 bp, Artificial Sequence
  primer
cataaccgatggagagcgaggtgcagagttcgtagg

SEQ ID NO: 65 - DNA, 37 bp, Artificial Sequence
  primer
gtgtcctacgaactctgctactcgctctccatcggtt

SEQ ID NO: 66 - DNA, 36 bp, Artificial Sequence
  primer
cataaccgatggagagcgagtagcagagttcgtagg

SEQ ID NO: 67 - DNA, 37 bp, Artificial Sequence
  primer
gtgtcctacgaactctgcaactcgctctccatcggtt

SEQ ID NO: 68 - DNA, 36 bp, Artificial Sequence
  primer
cataaccgatggagagcgagttgcagagttcgtagg

SEQ ID NO: 69 - DNA, 37 bp, Artificial Sequence
  primer
gtgtcctacgaactctgctggtcgctctccatcggtt

SEQ ID NO: 70 - DNA, 36 bp, Artificial Sequence
  primer
cataaccgatggagagcgaccagcagagttcgtagg

SEQ ID NO: 71 - DNA, 37 bp, Artificial Sequence
  primer
gtgtcctacgaactctgccgctcgctctccatcggtt

SEQ ID NO: 72 - DNA, 36 bp, Artificial Sequence
  primer
cataaccgatggagagcgagcggcagagttcgtagg

SEQ ID NO: 73 - DNA, 37 bp, Artificial Sequence
  primer
gtgtcctacgaactctgctcctcgctctccatcggtt

SEQ ID NO: 74 - DNA, 36 bp, Artificial Sequence
  primer
cataaccgatggagagcgaggagcagagttcgtagg

SEQ ID NO: 75 - DNA, 37 bp, Artificial Sequence
  primer
gtgtcctacgaactctgcccatcgctctccatcggtt

SEQ ID NO: 76 - DNA, 36 bp, Artificial Sequence
  primer
cataaccgatggagagcgatgggcagagttcgtagg

SEQ ID NO: 77 - protein, 307 aa, Artificial Sequence
  wex L79I
MNSKKATLIGLTAVVLWSSIVGLIRGVSEHLGATGGAAMMYSVASLFLLLSVGFPKLGSFPKKYLLWGSLLFVSYELCISLSIGYANTGRQAIEVSMVNYLWPAFTLIAAIAFNRQRANWMVVPGFILSIIGICWVLGGDQGLDLAGMLGNVQDNPLSYGLAFLGAVIWAAYCTVTARLAKGKNGVTLFFILVALTLWVKFFFGDHRPMSFSLPAIVYLLLAAAAMGFGYAAWNVGILHGNVTVLAGVSYFIPVFSAALSAMVLHAPLPRSFWVGASLVCAGSILCWLATRARRASAAQEDAVADCL

SEQ ID NO: 78 - protein, 307 aa, Artificial Sequence
  wex L79M
MNSKKATLIGLTAVVLWSSIVGLIRGVSEHLGATGGAAMMYSVASLFLLLSVGFPKLGSFPKKYLLWGSLLFVSYELCMSLSIGYANTGRQAIEVSMVNYLWPAFTLIAAIAFNRQRANWMVVPGFILSIIGICWVLGGDQGLDLAGMLGNVQDNPLSYGLAFLGAVIWAAYCTVTARLAKGKNGVTLFFILVALTLWVKFFFGDHRPMSFSLPAIVYLLLAAAAMGFGYAAWNVGILHGNVTVLAGVSYFIPVFSAALSAMVLHAPLPRSFWVGASLVCAGSILCWLATRARRASAAQEDAVADCL

SEQ ID NO: 79 - protein, 307 aa, Artificial Sequence
  wex L79T
MNSKKATLIGLTAVVLWSSIVGLIRGVSEHLGATGGAAMMYSVASLFLLLSVGFPKLGSFPKKYLLWGSLLFVSYELCTSLSIGYANTGRQAIEVSMVNYLWPAFTLIAAIAFNRQRANWMVVPGFILSIIGICWVLGGDQGLDLAGMLGNVQDNPLSYGLAFLGAVIWAAYCTVTARLAKGKNGVTLFFILVALTLWVKFFFGDHRPMSFSLPAIVYLLLAAAAMGFGYAAWNVGILHGNVTVLAGVSYFIPVFSAALSAMVLHAPLPRSFWVGASLVCAGSILCWLATRARRASAAQEDAVADCL

SEQ ID NO: 80 - protein, 307 aa, Artificial Sequence
  wex L79Y
MNSKKATLIGLTAVVLWSSIVGLIRGVSEHLGATGGAAMMYSVASLFLLLSVGFPKLGSFPKKYLLWGSLLFVSYELCYSLSIGYANTGRQAIEVSMVNYLWPAFTLIAAIAFNRQRANWMVVPGFILSIIGICWVLGGDQGLDLAGMLGNVQDNPLSYGLAFLGAVIWAAYCTVTARLAKGKNGVTLFFILVALTLWVKFFFGDHRPMSFSLPAIVYLLLAAAAMGFGYAAWNVGILHGNVTVLAGVSYFIPVFSAALSAMVLHAPLPRSFWVGASLVCAGSILCWLATRARRASAAQEDAVADCL

SEQ ID NO: 81 - protein, 307 aa, Artificial Sequence
  wex L79N
MNSKKATLIGLTAVVLWSSIVGLIRGVSEHLGATGGAAMMYSVASLFLLLSVGFPKLGSFPKKYLLWGSLLFVSYELCNSLSIGYANTGRQAIEVSMVNYLWPAFTLIAAIAFNRQRANWMVVPGFILSIIGICWVLGGDQGLDLAGMLGNVQDNPLSYGLAFLGAVIWAAYCTVTARLAKGKNGVTLFFILVALTLWVKFFFGDHRPMSFSLPAIVYLLLAAAAMGFGYAAWNVGILHGNVTVLAGVSYFIPVFSAALSAMVLHAPLPRSFWVGASLVCAGSILCWLATRARRASAAQEDAVADCL

SEQ ID NO: 82 - protein, 307 aa, Artificial Sequence
  wex L79R
MNSKKATLIGLTAVVLWSSIVGLIRGVSEHLGATGGAAMMYSVASLFLLLSVGFPKLGSFPKKYLLWGSLLFVSYELCRSLSIGYANTGRQAIEVSMVNYLWPAFTLIAAIAFNRQRANWMVVPGFILSIIGICWVLGGDQGLDLAGMLGNVQDNPLSYGLAFLGAVIWAAYCTVTARLAKGKNGVTLFFILVALTLWVKFFFGDHRPMSFSLPAIVYLLLAAAAMGFGYAAWNVGILHGNVTVLAGVSYFIPVFSAALSAMVLHAPLPRSFWVGASLVCAGSILCWLATRARRASAAQEDAVADCL

SEQ ID NO: 83 - protein, 307 aa, Artificial Sequence
  wex L79W
MNSKKATLIGLTAVVLWSSIVGLIRGVSEHLGATGGAAMMYSVASLFLLLSVGFPKLGSFPKKYLLWGSLLFVSYELCWSLSIGYANTGRQAIEVSMVNYLWPAFTLIAAIAFNRQRANWMVVPGFILSIIGICWVLGGDQGLDLAGMLGNVQDNPLSYGLAFLGAVIWAAYCTVTARLAKGKNGVTLFFILVALTLWVKFFFGDHRPMSFSLPAIVYLLLAAAAMGFGYAAWNVGILHGNVTVLAGVSYFIPVFSAALSAMVLHAPLPRSFWVGASLVCAGSILCWLATRARRASAAQEDAVADCL

SEQ ID NO: 84 - protein, 307 aa, Artificial Sequence
  wex L79S
MNSKKATLIGLTAVVLWSSIVGLIRGVSEHLGATGGAAMMYSVASLFLLLSVGFPKLGSFPKKYLLWGSLLFVSYELCSSLSIGYANTGRQAIEVSMVNYLWPAFTLIAAIAFNRQRANWMVVPGFILSIIGICWVLGGDQGLDLAGMLGNVQDNPLSYGLAFLGAVIWAAYCTVTARLAKGKNGVTLFFILVALTLWVKFFFGDHRPMSFSLPAIVYLLLAAAAMGFGYAAWNVGILHGNVTVLAGVSYFIPVFSAALSAMVLHAPLPRSFWVGASLVCAGSILCWLATRARRASAAQEDAVADCL

SEQ ID NO: 85 - protein, 307 aa, Artificial Sequence
  wex L79P
MNSKKATLIGLTAVVLWSSIVGLIRGVSEHLGATGGAAMMYSVASLFLLLSVGFPKLGSFPKKYLLWGSLLFVSYELCPSLSIGYANTGRQAIEVSMVNYLWPAFTLIAAIAFNRQRANWMVVPGFILSIIGICWVLGGDQGLDLAGMLGNVQDNPLSYGLAFLGAVIWAAYCTVTARLAKGKNGVTLFFILVALTLWVKFFFGDHRPMSFSLPAIVYLLLAAAAMGFGYAAWNVGILHGNVTVLAGVSYFIPVFSAALSAMVLHAPLPRSFWVGASLVCAGSILCWLATRARRASAAQEDAVADCL